European Patent Application EP 4 151 740 A1, published March 22, 2023. Title: A BIOASSISTED PROCESS FOR SELECTIVE CONVERSION OF ALKANE RICH REFINERY STREAM. Applicant: Indian Oil Corporation Limited. Application EP. The sequence listing filed with the application follows.

SEQUENCE LISTING (2 sequences)

SEQ ID NO: 1 - DNA, 2880 bp, Candida tropicalis
  source 1..2880: mol_type = genomic DNA
catatgcgctaatcttctttttctttttatcacaggagaaactatcccacccccacttcgaaacacaatgacaactcctgcgtaacttgcaaattcttgtctgactaattgaaaactccggacgagtcagacctccagtcaaacggacagacagacaaacacttggtgcgatgttcatacctacagacatgtcaacgggtgttagacgacggtttcttgcaaagacaggtgttggcatctcgtacgatggcaactgcaggaggtgtcgacttctcctttaggcaatagaaaaagactaagagaacagcgtttttacaggttgcattggttaatgtagtatttttttagtcccagcattctgtgggttgctctgggtttctagaataggaaatcacaggagaatgcaaattcagatggaagaacaaagagataaaaaacaaaaaaaaactgagttttgcaccaatagaatgtttgatgatatcatccactcgctaaacgaatcatgtgggtgatcttctctttagttttggtctatcataaaacacatgaaagtgaaatccaaatacactacactccgggtattgtccttcgttttacagatgtctcattgtcttacttttgaggtcataggagttgcctgtgagagatcacagagattatcacactcacatttatcgtagtttcctatctcatgctgtgtgtctctggttggttcatgagtttggattgttgtacattaaaggaatcgctggaaagcaaagctaactaaattttctttgtcacaggtacactaacctgtaaaacttcactgccacgccagtctttcctgattgggcaagtgcacaaactacaacctgcaaaacagcactccgcttgtcacaggttgtctcctctcaaccaacaaaaaaataagattaaactttctttgctcatgcatcaatcggagttatctctgaaagagttgcctttgtgtaatgtgtgccaaactcaaactgcaaaactaaccacagaatgatttccctcacaattatataaactcacccacatttccacagaccgtaatttcatgtctcactttctcttttgctcttcttttacttagtcaggtttgataacttccttttttattaccctatcttatttatttatttattcatttataccaaccaaccaaccatggccacacaagaaatcatcgattctgtacttccgtacttgaccaaatggtacactgtgattactgcagcagtattagtcttccttatctccacaaacatcaagaactacgtcaaggcaaagaaattgaaatgtgtcgatccaccatacttgaaggatgccggtctcactggtattctgtctttgatcgccgccatcaaggccaagaacgacggtagattggctaactttgccgatgaagttttcgacgagtacccaaaccacaccttctacttgtctgttgccggtgctttgaagattgtcatgactgttgacccagaaaacatcaaggctgtcttggccacccaattcactgacttctccttgggtaccagacacgcccactttgctcctttgttgggtgacggtatcttcaccttggacggagaaggttggaagcactccagagctatgttgagaccacagtttgctagagaccagattggacacgttaaagccttggaaccacacatccaaatcatggctaagcagatcaagttgaaccagggaaagactttcgatatccaagaattgttctttagatttaccgtcgacaccgctactgagttcttgtttggtgaatccgttcactccttgtacgatgaaaaattgggcatcccaactccaaacgaaatcccaggaagagaaaactttgccgctgctttcaacgtttcccaacactacttggccaccagaagttactcccagactttttactttttgaccaaccctaaggaattcagagactgtaacgccaaggtccaccacttggccaagtactttgtcaacaaggccttgaactttactcctgaagaactcgaagagaaatccaagtccggttacgttttcttgtacgaattggttaagcaaaccagagatccaaaggtcttgcaagatcaattgttgaacattatggttgccggaagagacaccactgccggtttgttgtcctttgctttgtttgaattggctagacacccagagatgtggtccaagttgagagaagaaatcgaagttaactttggtgttggtgaagactcccgcgttgaagaaattaccttcgaagccttgaagagatgtgaatacttgaaggctatccttaacgaaaccttgcgtatgtacccatctgttcctgtcaactttagaaccgccaccagagacaccactttgccaagaggtggtggtgctaacggtaccgacccaatctacattcctaaaggctccactgttgcttacgttgtctacaagacccaccgtttggaagaatactacggtaaggacgctaacgacttcagaccagaaagatggtttgaaccatctactaagaagttgggctgggcttatgttccattcaacggtggtccaagagtctgcttgggtcaacaattcgccttgactgaagcttcttatgtgatcactagattggcccagatgtttgaaactgtctcatctgatccaggtctcgaataccctccaccaaagtgtattcacttgaccatgagtcacaacgatggtgtctttgtcaagatgtaaagtagtcgatgctgggtattcgattacatgtgtataggaagattttggttttttattcgttcttttttttaatttttgttaaattagtttagagatttcattaatacatagatgggtgctatttccgaaact

SEQ ID NO: 2 - DNA, 1800 bp, Candida tropicalis
  source 1..1800: mol_type = genomic DNA
gtgggttgctctgggtttctagaataggaaatcacaggagaatgcaaattcagatggaagaacaaagatctaaaaaacaaaaaaaaactgagttttgcaccaatagaatgtttgatgatatcatccactcgctaaacgaatcatgtgggtgatcttctctttagttttggtctatcataaaacacatgaaagtgaaatccaaatacactacactccgggtattgtccttcgttttacagatgtctcattgtcttacttttgaggtcataggagttgccactgagagatcacagagattatcacactcacatttatcgtagtttcctatctcatgctgtgtgtctctggctggttcatgagtttggattgttgtacattaaaggaatcgctggaaagcaaagctaactaaattttctttgtcacaggtacactaacctgtaaaacttcactgccacgccagtctttcctgattgggcaagtgcacaaactacaacctgcaaaacagcactccgcttgtcacaggttgtctcctctcaaccaacaaaaaaataagattaaactttctttgagcatgcatcaatcggagttatctctgaaagagttgcctttgtgtaatgtgtgccaaactcaaactgcaaaactaaccacagaatgatttccctcacaatcttataaactcacccacatttccacagaccgtaatttcatgtctcactttctcttttgctcttcttttacttagtcaggtttgataacttccttttttattaccctatcttatttatttatttattcatttataccaaccaaccaaccatggccacacaagaaatcatcgattctgtacttccgtacttgaccaaatggtacactgtgattactgcagcagtattagtcttccttatctccacaaacatcaagaactacgtcaaggcaaagaaattgaaatgtgtcgatccaccatacttgaaggatgccggtctcactggtattctgtctttgatcgccgacatcaaggccaagaacgacggtagattggctaactttgccgatgaagttttcgacgagtacccaaaccacaccttctacttgtctgttgccggtgctttgaagattgtcatgactgttgacccagaaaacatcaaggctgtcttggccacccaattcactgacttctccttgggtaccagacacgcccactttgctcctttgttgggtgacggtatcttcaccttggacggagaaggttggaagcactccagagctatgttgagaccacagtttgctagagaccagattggacacgttaaagccttggaaccacacatccaaatcatggctaagcagatcaagttgaaccagggaaagactttcgatacccaagaattgttctttagatttaccgtcgtgaccgctactgagttcttgtttggtgaatccgttcactccttgtacgatgaaaaattgggcatcccaactccaaacgaaatcccaggaagagaaaactttgccgctgctttcaacgtttcccaacactacttggccaccagaagttactcccagactttttactttttgaccaaccctaaggaattcagagactgtaacgccaaggtccaccacttggccaagtactttgtcaacaaggccttgaactttactcctgaagaactcgaagagaaatccaagtccggttacgttttcttgtacgaattggttaagcaaaccagagatccaaaggtcttgcaagatcaattgttgaacattatggttgccggaagagacaccactgccggtttg